European Patent Specification EP 3 761 780 B1, published June 19, 2024. Title: COMPOSITIONS AND METHODS FOR PRODUCING TOBACCO PLANTS AND PRODUCTS HAVING ALTERED ALKALOID LEVELS WITH DESIRABLE LEAF QUALITY. Applicant: ALTRIA CLIENT SERVICES LLC. The sequence listing filed with the application follows.

SEQUENCE LISTING (36 sequences)

SEQ ID NO: 1 - DNA, 2001 bp, Nicotiana sp.
cttttacctaaacttaaatattggccttatgcacgggcatcaactcgcgtattactaagaagaaagaagaacggctcctcgtctcccatgtcggcctctggaactcttaatataaccgccgacagacaaaaccggctggtctctcactgtttcttatcctcagaattattatgaacataaactaaagtacctatctcttgttttctcatttcacaccatttttttcttcacttcacacttggtctcaatcaaataaaaaacagcaaccgccttagcttgttgtcttcttcactactccacttgtccctagagttccccaaaaatatcaagctaagaaaaagttaactaaagaagagaatatatgggagctgaggtttctttcataagctgaccgactctttatttggcggcgcttattttatttattacttcaaaagaaaagttctttttgttttccttttttataattttcaactcccaacttgtgtgtgttgtctaaatgtctatatataaatatgtatataacggtttgtttaagaaacttgcattggtactggtttgttcttgtcaaccttcttgactagtatatatattgtaaacttttgtgtctctgtattggagatttttgtttgagttctctttttgaatattgcatgtgtatttacaaggtggcgaattcaagagacaaaatatctaacaggagaagacatgaagatagggatagagatgataattataatgtgttggaatcgatgttttcgggtaatattaatagggaacaggagatgtctgtaatggtttctgcactaaaacatgttgttgctggtgaagatagattgaatcaccaaatcttgactgatgaaaatggtgcagctgagaataatcttggttcaggtttttcttcagtttcttggggggttggtgagaaaagaggacgtgaacaacggcaaagtagtcagcaattcttacatattggaagttctgatatgagatcatcaggtatttttattttactttacttttttttttgaaaaaaatgacaccgccgtaaaaataataaccgaaaaaagtgtataaaatttgtataatttttgcgttatatatatacattctgtatgttatatacaaaaattatacaaatagttaacaaatttgtatataaaaattatacaaattttatacatttttcggctaccacatataaatagtttctggcgccggctaaaagtgataataccccttttttccttaaagttttggattttcttttagtttatgttgtgttttcagtgggtattttgaaaacataattaactagtggccaatgtagcattatacggattcaattgaatccatagctttcgaggcataaaataaatttatgtgtaaaatttcattaaagttataagatatagtagaatttgaacccatataacagatatgaacccataactttaaaaatacaatatgttcaatgctagaatcttaaatgttcaacccacaaaatttaaattttggatccgcctctgattattaaaagtatattttctctaacggtttaattaacatttagataagatgatcaaacattaatactatgatattagagtgggtataagttccgggctgaagcttaaatatttagatgaaacagacacacaattcaatagtttggatgtgttgcaggaatcattattgctaaataacagctaaatgtagatgagaataaatggattaaaagatttggttgatcttctatgtgagttgtattcattctgcattttatttagaagtaaattgctgcagatgcctttgtttttagttttgattcttgccattttctccattaaaaaaatgcacttgaaacatacaatataaatcaagtgtgtgacttttcactatattgatttttagtacattattaatgaaagatacaattaggtggatgtgtacgtgcttcattatcacattttcattattttgaatagcagattttacaca

SEQ ID NO: 2 - DNA, 2001 bp, Nicotiana sp.
ttgtttatgttgtatgtattggtttagtgagttatgatataatgttttcattgaaagtgtgacatgatacgagtattttcaaatggacgtgagttagcatttcagattttcacttcatttgtcctatttatattaaacccacaaaatgaaaatacccgtatttatgtttatacactttcataaatttcaagaatttagacaaaaagatttagctttaaaattttgatatggtaattttgtacgctattttaaaactattatgttaatatttatcctcttttttaaatttcacaaaaataaatacataaaatatttatttgtaatttttgtttttcttttaataattacattttaaaatacttagttatggatatacctcatagggggtataattaagtgtatgatttttataatatagggggtgtcagtgtttgatcttaaaatacaaaagggtgtatccgaaactgaatcgtattatatgggtgtttagtataattaacactattatatataagtaatattgatatttaaatctccgcacttaattaaatactgtctcgtaaaattaacgtctatgtgtactgacaataatgtaatatttttttaaccttgttataataggtaatttgtattatttttgaattgatatctcttttttaatgaaaggttacatataattatcatttagatgataagagcgtgcataaattcattaacaatatctaacatatagagggatgaagtagtactattaattttctaaaaaatgagaagcaaaaaaggaatattcttctatgtcggcctctagcttagctaagaactcaacgccgactgacaaacaactcctaaagcggctctaattttttctctctaaaatattcttatccacatataatagatctcccttcacacttactaatactgctgtcctttattctcttcacattttgtccaaaagaaataatgacaagtcaacaataaaaaacaatgttttcatcaacaagattaatctctccttcttacacgcaagcaaagatggatctagaatttgcggagatacatgaacaaactgttcaactagtgccacccaggggcgaatttataggtaaatatatggggcacttgaacctattatttttccatcaaactaagtattttatgtatatattttttagaattggtctagtattatctgctgacactcatgctccaaaaaggctaaatggtgcacttggttgaatattgaattatttacctaaaggactacgaatcgaatctcacttaatactttttttttcctccttttttaatagtgcactcatattataaaaatcctatatccgcctatgatgtcaccatcaaacttttgattttaacggttataagtaaattatatcatcgtttttaatatatatagacaaatattttaaaaaaaattgccgatgtgtgacctctatctcctagcataggtccgccaacttggagagaagaatacaaattaaggaagctcatgagctgactagccgactctatattcttgtctttattattttacaaaaaagtttgactttacttttttgtttttttgttttaagtaaattttcaactcccaacttaggttagtctaagtctctatatatataacggttggttcaagaaagcctaaaaaagagggggttagctggttggtataattagtttgttcatcttgtcaactttcttgaaaagcaaaagtttttaatattttgttttcctctttttgaatcttgaagtttgattcaaacttctcattttatagaatactctgttaagactttttagttagtatagtatactagctatatactagattaacttttttttttttatttataaagtcccttaatttagtgaagttttgttacatgtgtatactcaaggtggcaaattttagaaacaaagccatttataagccaataagagatgatgtgatgttttctgggattaatagagaagaggaga

SEQ ID NO: 3 - DNA, 2001 bp, Nicotiana sp.
aggagcgttcaaagtttagatgatttattatggtatatgtgcatttttcaccacttgttgccaatataatactacattttcctctcgagacgacaaagaatgataatgaagataccttttcttgctgaagattttgtcagtatactgcaactgattttagcaactttgctcttcatattataagtcaattatatactgtcgaatctttctattgtttaatcagtcgcccctcatgcatgtaaattaaagtataatatatataaagtataacttgaatgtggatttttcccccacatatataataaaacaatgaaaggaaaagatctatatatgtgtctttgatttttagtgggccaaacaaaaaaaaaagaagcagcaatatgtcagtattcaggagaaattcaaaaatagtcagatttacaactgatcattcaaaaatagttcagtttcaaaagtaatcaaaatttagccacttttcatgtaaagataaaaaagagcgaaaatattgttcaaaacccgaaaaatacgccagtatattatactggagttcaagtataagtatgcttgaactccaacatattatattggagttccaggataagtatgttggaactccagcataatatgatggagttccaacataagtacactagaactctagcataatatactggagtttcagcaagtataattgtccagtataatatactggagtttggagcacaagtgctccagtctccagtatattaataatggagtcagcaaagtataccggtccagcataatatgctggagttcatacacaggtgcaccgaaatccagtatattatgctggaccggtctctgttgcagcaaaatagtggctatttttcattgactttgtaaacactgactatttttgaatgaccagtccgaaaactagctataccgtgctatttttacatgaaaaacggaatacatactataatatatcatgttgtttatataaattgaaaagacgaataactcgaataaaaattcaaaatagtcaaatcgatcaagtgtgtaccatatttggaacgtgtaaatagcaaatctctatgtcggtggggcaccctctctgttataatacagctccagataagtacagtctaaattgaagtttcaacttgtgttaaaatatttaatctgatattatctgcatgctacataattattgtacgagcttggactttggggctcatgcttttgtccttcgtttcgagaacgcaaataagttcggtgcactaagctttcgctgtgcgcgggtccggataagggtggaccacaagagtctattgtatatagttttaccctacatttctgcaagaggctgtttctatggcttgaaccggtgacctcctggtcacatgacagcaactttatcagttactccaagactcccttttacaaacttcacttattattacgcaaaaagaaaagaaaattgttgtggcttagttggataggacactttatttgacgcaattcttgaaatggtaaaatacacttaaaaatcaagcattttttatattctctgaatcaggtcaactattcagaagtgtttccaagttgtcatacaaatactttttccccccaagttgcagaggtcataacttaacttacttgacgtcaaaaatttcatttaaggtgttcaaacttaaaataagtaaaaaaaatctccgataaagggtgtttaatatatcttatatatcattaaaatttaatattttacctatatatataatataattttcagacaaagggtggtcagttgaccaaacttagggctatgtaccttcgcccatcatgactatatatatatatatatatatatatatatatattgttagtagcccttcaaagttgcataattattagagagaatacacatttaaatattgaccaaacttgtctataaatttggatatttttgctactttaattttctgaagcaaataagaaagaagatcatttgagaaa

SEQ ID NO: 4 - DNA, 2001 bp, Nicotiana sp.
tgtcgcaggagcttatccaccaccttttgtatgatattttcttttagttggttatttgatttgtccttttctctatccaatcgaacaattataagaaatgcaccaatattacttttatctatcccaatttatgtgatatttttattttctgagattcaaattttttaattttgattatatacttagacataaaatcttttaacttttccgaaataaaaattacatatttgaaaattacgtaaaaagtactataactcacaaaaaatattaattttaaactatttaaaaatatatataaaaagattacagtcaaataataactcgtttgactctcaagatacggataccgtcacataaatgggacgaaggtggtatattgagtgtcctttcataaacatagtactagtattttttgggaagctccatgaaaatgatattttttaatttttattagtttattttaattttttattttatccataatgatatttttataatgacataaatattttcgaacttagtaactgttgctcaaagtttgcatatttattaaaattcaataagcaagtgcaaaacgtttattgcaaactcaaaaaattaaatgagttatttcataaaatttaaatcttgaatttgcatacagtaacttatttaaaattatatattttaaattaatttttaatatgtacccgtgggagttgggtcggaggaagtataatggagacagaaccagctaagataatcaataattatactaaaaggaatttagtactttctttttggtgttctctctgtttcagtttatgtgaacctattcttttttagtccgttaaaaaaaatgatctttttctaaatttagtaataatttagcctaaacttataattctacccttaatgagaaacttttataaccatacaaatattctgagtcttctttttaacttgtttagtataccaaatttcaaaaatctttattttttttttaaattttatgctcaatcaaatatgttcacgtaaattagaacggatgaattatcacgtaactaatctaagtaatcacagttgtcttacatcaagctggtcataggtaaggggaaacactaattccaagaagtcgtaacgtgacctaaattaaaactgccaccctttggacaaaaacaaagggaacccattttgccccattgtgacaaccaaatgacacaacatggcatatattgtgacatacaccacccaatcaccaaatccaactaataaatgtcttactttttgcatctaaggttgtaacctaactaaatataatgaataaaatttgtgaaagattaggattcaaatatataaatagctaaaattatagatttcttttttttctatttaaatagcttatttggtcacatttctaaaattagcttattttttttaaaaaaaattatttttctcaaaagttatttaaaaaaaatacttttgagaagcagtttgtatttgagtaatcaatttgaaaagcatttttgagtagcaattaatctttggtcaaacttttaaaaattatttgtaaatatatatatatatatatatatatatatatatatatatattgaacaaaaagtataaatattttgtgtcgacacttgcgacaaatagatgggtcacattcaatccaacatctcattagcttctactacgtgtttggattactcccccaacttgatggctgattgatcatcgaatttttgccacactatcacttcttatggtccaaatacttctcatacttttctatacataaaattcttcaaacccctcgaaaggtcaattatcaactttcacgtgatcttggaaacttgcaactttcttgccatgcattgtcacttgcttgaccaacttgcatcacctttaatattagtaataaaatttttttactttccaatctcaagatctataaatagaaagttttctttccttagttcttgtttcactatcaaatgaagaggcaaagaggaaaga

SEQ ID NO: 5 - DNA, 2001 bp, Nicotiana sp.
ttttatacccatactcgtgatcatattagcgatccccctaatcgtagtgacggccactcctgcaatttcggacctttgtacggtacaatagcgaatagggctcctaaaaaacgtaaacctgtaaatgataaagataacagctaaaaaaatgcaaccatcctttgaaacaatattttttttaaaaaaaaaaaaaagttcttgcatgcaaatttaacttcgtatactaatctccaatgcgatttagaacttaaaaattactattcctaaacaattagaaaaactgcatttcttaatctaaggatgttttgtgtctgtcctattgaaacaactttagactacagatcgttaaattgtaatcaaccttcttttagtgtaaactgacgcggctttaccctttggtcagttaaataatccttacatttggtaaatgcttatatttactcacgcgattaagagtaatgacctcgcaaaggtagagttcaactgcacctcactttgtattctttgaaatagccctcaaacattacgtcaatgaaataacgatatgatctcgattttgaatttctgagtcccaggttagtatatatataattacattcctattatcatggcagatatttcaaaaaaaagaaaaaagattaaaaaaagaaagaaaaactgacctagaaatatctccagtccgcttcctagaaatataatgcatgaacactagaagataggacatttaagagagtcacatggttgtttatggcgagaaatattgctaaaaataaaaaaaatatgatattatatgtcacataaagttggataatgtaaatgttggaggataaaacacttcaagcccaatcataggccgactggtgaatggctgcttaaatttcaaattgatttacaccctaccaaatacaaaaatataaactctttggtattgttactatttggcaatcaatcatattcataattggcatgtgagttgaagctaattgatgaagcgaaatttgatgcgtgagtagtctctttattgcaccacactaactgttgagatattttgctcaacttatttgaagaaaaacaaaaataaaaatgaactctttggacactttcaatctttcattgccatttatcaagataatctgatgtaactaaaaaaataataggaccagtacccaaaatccagatcttttcccagcaacaggaaacctttatcaaattttagtccccatttagactacctaatcaaagaagatactctgcattcgacttaattcacgcacattgtcaataagacaaagaccttagcgaagccaaccaaactctttcttttactttttcatattgctccatcagttttaatttatatcacacagtttaattcggtatgggatttaaaaaaaaacttttaaatcttgtggtctttaaagtataaaagataaaagttttgtggagccataatatttgtgtgactataaaaatttctaaaataaaatatttataattatattattttcaaatatagaatatataatttttttggaacggactaataaaagaattgtattatatactatatcaattgaaacggagggagtagatggttatccgcacgcatctttagtagtgacagttattcgatcttataataggttggcctatgcatgctgatgtattgtcttttagtagctacatattgagttgaattaccttttaccatgcctgcgaccccatgcaaacaagagcttaggtcctacgaggaatgtccttctcagcacgccagatgcacatacatgaaccaaggcaaaaaagcaaaggaaatttaacctttttgccattaattacatttaaactggactagctcattcccccagctctcttacccacaagctccttctataaattcagaaaccaactgcaccccccacattcatcataactcgatctaactttagttattgagagacaaaccaattacagaagcttaatccttagagaaattaagagaga

SEQ ID NO: 6 - DNA, 2001 bp, Nicotiana sp.
gaattttggtatttttcgaaaatttgaaaaactccaaaaggttatttttcaaaattttcccttcaaatcactcacaaaatttcaaaaacagctccaatttatattcatatccaaacacaactataattttcaaatactattttgaaaaataattttacttttttccgaaattttacaatttttatgtccaaacacccacgtagttctttcaataaaatttctaacatgttatggcaagacatgtaggacgagagttgatgtttttttttcttttgggcttttcaaatcgagttctgcaatgaattggatttaacaataatagccatctatgactagttattaaaagaatttgataccagaccattttaaccagatttgtcatttgtaggaatttgggcttttgtatttatacccgattttggggtcacaattgaagctataactacttcgcaaaaaaacttgcaaacctacccactttacaattaacttcaggcttatcgggtctgaagttaaaaaaaaatagtctgaagtgcaacgcacttaaggccaattaagtctaaagtgtaaaaactaaggccaaatatgtctgaagtacaaccaatggttttatacatttaagaccaaatagatgtgaagtgtaaccaatagtttcacacacttaaggtcaaaaagtctaaagtgaaaaatttgcacttcagacttaaggacaaataggtcagaagtgcaaccaatagtttcatatacttaaggccaataagtctgaagtgaaaaaattgcactttagatgcacttaaggccaaataggtctgaagtgcaaccaacattttcatgtacttaagaccaaagaggcctgaagtctttggacttaagtgcaaattgcccaaaaataaaaatttgttcttcgaatttttacaattcaatacacgatttaacacctaaatctactccaaatgagaaaaataaagcttcgaaacagcttaccactgtaaaacatcataaactaccttaaaatatgttcacaaaacaccatataaaatcactatataagaagaagaagaagaatgaggaggaggaggcctgaagttgtttaaactttggatactacttaaaaaaaattaaaaagtgggtataggttaaatgaggaggaccaaatagggcactccgtaaaatttttacatagtaattaccggtcaagaaagttaagtaagagggatgccacactctattgagattaccccaataaatcaccgaactccactgcttcatcaaactacagaacatggggtctttctctctctctccctccctccctccctccctctccaactctatctccctcaatacgcacaagcagtactttttcattttactttatatttgtgaaggggaaccttgaaacaattataaacttatttctatgtgacatgtcacggattcgagctgtggaatcagccactaagactagcattagggtagactttctacatcacactccttagggtgcggccattatcgcacctgcatgagcccggaatatcttgggcgccgagcttcccttttttatatttgtctgtatttttgaataaaaagaaacaaaggtaggaagtgtttaggaattttatttcttatggataatgtataaaatcctccccggcctattaccatattaccaactacacactttttttttccgggaattctattaccccatgaactattttaaagtataataaacaccaccctaagtgatgatgtggcatagagagtatgcacactctcttaagggcaagtggaagttacaaaaataattttaaaattgattaacatgtacaagtgtcatcttttgattggacattacacaattaattatatctaatttattagtctccttcgtcttctaaatctcttcttgcacgaacaagggagacatcgtttcagcggcgaaatgcctgagcgaaaatccaatacaacgcaaatcaaccgagaaatcaaaagcagata

SEQ ID NO: 7 - DNA, 2001 bp, Nicotiana sp.
gttttagagagtactttggcaagaaaaacaagtgtgagagatcacccaaaacatcatattttcttcttctctttatttttctggcaattttgatcatgaatattttcatagtttatttacccattgtcatgagtagctaaatcctttgtctagggttttgatggaacctattgaagaatgaacttcttgattatgttaatatagtttgccagtttaatctctatttgttcaactacgtgtttgttgtagttatttgacaggatcctcaattagctgtgcctatttggtatgcataactcgggagagagtgcatatttaggtaattgttgaacaacatcactcccaaagtataagagggatctataactgcgggtttaaaggcggaattagggataacgaagtcttgggtgcaatctaaagtgaactgtaataaacaaagccaggtagcgtatctcgggagagtgcgtctagtaaattatcgtgattactcgggagagattcacggtaaaaatagtgttcatggttgatagagatgtgttggtaaatctatatgaaacataaacagaagggattccatcaatatgggaaatcactaccttagaaccttctcattattgttcacaacttaagcatatttagtttacaactatttattgactttcaatcttagttattaaatataccatcgactgttattcacaacatttggggaagttgattctaaagaatttagtaagtccaacgaaagtaattgataggttaattctctgtggattcgactctcgacataaatattcagattatatttgcaacgtgtgcattgtccttttataaggtatagttgggcatgatcactaatacttacattattttttctaatacttgccaaatgaccccaacaaattttcagtctaaatggccggctagtcgtaatagtttaacgtattttaaacgtgcgaaaggggcttcttgactttatcattttatggtttcagccggtagatggggacaacctacaaattatgtggccaaggggacaacccaaatgtgaaaaactaattattatttcgttcatttcaatttatgtgtcttattttattcaattttttttatctttttaaatagtagtaaatttttaataccaatgtttgtattttactcttaatgacacccgttataaggaatcatatggcaatatatatatatatatatatattgacttgaagagtactttttatagcttatacacacctttaatttaaggtaaacaatattaaaattcattttacattttagtccatttaagctatacccacctttcatttaaggtaatattaaaattctttttacattttagtccagttaatctagaacatatcagatgaaactgatcagagagtaacgatttaaattttctctgaagcagcttcagtcatatgaggcgcaatatcaaatttctcctttttggctaacgaaataaaaataaatgcgttagaagtctctggtccgaatagtagttgttcgtttaaaacgtttataaatttaaagttctactgtagccgaacacgtttgtgtataactatatatatagacaaaattaatagtcagccaccaaatcagtaggttaatcttctaaaatgaggctatttaactaaagctatagtctatgtacaatttcaggcaaccctatgctacttcaacaaccttggtccccttgaagatctcaatatcccaccttatcaccttatcttgttgatgctacaacgtattgtatttgattcttttacttttatcctgagtagtggatttatcggaaacagtctctctaccatcacaaggtaggagtaaggtgtgtgtacactctaccactcccaaaccccactttgtgggattacattgtctttgttattgttgttgttgtcgtcgtcgtcggcggcttgaagttctcattatattagcagccttaagttcttgttcattcttgtttcttatactgccaga

SEQ ID NO: 8 - DNA, 2001 bp, Nicotiana sp.
tttaataagcagcggtttatttccgggcgaaaagggtaagtcggcccctagcagtgagaaaccaaaaagaaattgttccttatattgtgcgcatgtcaacttttttggcttggcttgtagacgtatacacgtggaattaatgagagaagataataggagtattatagtagctaggtacatagtatttagcaaatctttcatggctttgacttcccacgaaattaaagcagtaatcttcataagctgcatattatctccattcttatcaccttttgtacctacccacataaagcccgactgtttggttggtcaaaggtcgaaatatctatgcaacttggccaatatgctttctatataataaaatatgcatggcctaccatttaatttgtatagcaacaaaatgtggcaaataaaaaccctaccagtataatttctgagctttcaacctaaattaaagaagtctatatcatgctcagcctatatattttgaccatcgagagcaaaagcatgacgatgattccttgtatttaagagtaccgtggcttaattgttaatgaagtgagtgataattatcggagattagagtttaaattattagcagtagttatattttatctgtctatgttatggtggcaaagttaccaaattcatttgctggttgaaggtaattaccgatgtttaatttgatgaaataatcgaggtgcacgctaacagtaggtcattagcctcctataatgctgaaaaggatgccctaaacgtattctaaatttctatgtcataaccatacgtcaagggttatactattatactactacagtccaacactcgagaaaaattaggacattgagtttttattttttatttttaattggcgaatactgttaagttggttgcaaattatatactatctttttcttgttaaaaaaatacacaaatatagagacaaattgactaaatgcaatcaaaccaaacgctatatcaaacagaatctgctgtatttaagacttattcaaagttgagatctcaacatctcagccttaaaaagttgagatgggtaatattggtttttaaataattatatgacaaaaaagaggtaggttgtttattatataaagatggatggtgattctccagatatcttttggcaaacataaattaaaccaaaattcaacgccttaaaggattaactaaggctccaaatgtgaattgcgtaacgctgcatgtccccaaaaagtgaggtcggcattagctgaaatatcttttcaggattatcccaaaagaaaatacctagtcacccccggtacttataccaaatcgagcaatttaaatctaaaaattataattaaaattgaaaatacatatcacttaatcttaatcaagtgataaaaatttacacgtcatatatttcttgaatttgtggtaacactattaaaaaaaaactccgcctaaatgatctaaagtcaaatttgaccccaaaaaaaatctaaactaaagtcaatgctccaactcaaaccggcgtcggatacggggcgtcactggtcagtcctatcaggactcgtgagacttgtaattcttatccactaattctcataaattcaatcatattacgttatatttttagaaaacccatataaagatgaagtagaattagaatttaatatgttttctatatatagatccgaaattagaaaagaagaaagggcagagatctgggttcttttatcattgatcttctgttttccaattgtcttaattcagtagctgtcatgcatgcactagataaaagttatcactaattttcagtgggttccacaagtgcatgtaagtcttaggattttactactgctacttgtttggtgacttttatatatattgtttcatagatatcaagcattgggtgattataacaacaaagatttcagattcgactaattcaaattcgtgtcggataagattatataaggaattgagaacataaaataaggatctttcattgaaaaa

SEQ ID NO: 9 - DNA, 2001 bp, Nicotiana sp.
tggtatgaaatttgaattgcattgagtattcttcgtgttgctgttgtgtgtttactttgagactatgagacggtatcccgagagatccccctgcatgtttactttgggactacggatttgtattccgggagatccccgtgcacttttatattggaactacgggattgcacccggtagattcccccaatattgggtatttatatttgggactacggatcggtattctgggagatccccgcgcactatgagttggactacgagacagcacccgggagatccactggatatttatatttgggactacatgatggtatcctgggagatccctggttgttatctctgtgttaagttgtattccttctgtgattatttggctctgttatagttgttgttatttttactatcctgtgttacttcttattgtttgcacttaattatattgtcttattctatattgttataccttgtttttcatctaaactcagtagggccatgactttcctcgtcactacccgaccgaggttaggcttggcacttactgagtactgctgtggtgtactcatgccctttctgcgcatgttttttcatgtacagatccaggtacttcgactcagccttactatccttaaggcgaggcgattctccagagacttcaaagtatatcttccgagtccgcaaaccgagaagtccctttctattctcccatatagtattagcccttctgtatttacttttgtttaaacattctggagttagacacttgtagttatccaacagcttgtgatttcattagattccgggttttgggaaatattgtttcagttcgagagtttgtattgtatatgtcgagcggcatctaaacgcttcattatgttatttctgtagtttttgactagttttattctgttattttctgtttccgtaatttgttaagcttacctagtcgtagagattaggtgctgtcacgatagttcacgaaggacgaactggggtcgtgacaagtttacttagattataggagtttatgggatatctacagtattttttttttatatacattttattgattaatatgatagacagttcaagaataaaagttacaccgctagtacgtaagaaatttattcttaacaaatttaatgaacccaagttgtggttgaaaaaaaaagttgagtttgaaaaaaaaacatttgtatcaagttggggttgaaaaaaacaaattgaaccaagttgaagatgaaaagagaggagagttcaaaaaaaaaaaaaaagaaaaaaaaaaaaaagaggagaattcaagttgaagatgaactctttaaccactgtcttcctctttctctctcctggtataaaccgacattctttaaggagttcgaaaggtcgaaagcagatgcatgtaacttcatcattttcagtcaaagtgcaattaacggtgggaacatatctctctgagtcggccgctgtattgttgtttttttggcaggcatcaaatctttcttttttatttactatttaaagaaatttaataaaaatacaaagctgagtatatttaactattctttgtacaatatagagattgacaccaaacttcgtgcatgatctattagcagaaagtagcacgaagattcaactattctcttcacggctgttcaagtttgaattttcctccttatattatatagccgtttgtaagggaatttttatcagttatctgtaaaaagaatcagttgtctactttgtgcatgtgctccaaatcaagtaaaataccataagggagcccatcaattcagaaatatacgatttgggttggtcttatttttgtgctacgaaaagtgttcgacgaaattgattttgtcagagttcaaagtcggtggcttcagattctgcagaaacggtgttgtgttgaagaaaagctgaaaagggtatttataattcaccaaaaaagcatctgggttggtgttattttgtcgtaattttgtctagtttgaagtgggtcgtaca

SEQ ID NO: 10 - DNA, 2001 bp, Nicotiana sp.
acaacaacaacattattattaaaaacaactgcggaggcatgattgttgttgttgttattattgttttacgtaatattgttaaaaaacaacttcagatgcatgattaattaagctaggatcgcagtaaaatttcataagtgggatctggagaggatagatcagcgtacgcaaatcttatccctacattatagaggtagatgggttatttccgatagacactcggctcaaagaaagcgattccaaaacatattcgaagaaaggaaaaaaatatgtcgaaagtaccgacaaaaataatacgataatactaataaaagaatagaaaaaaaaaacaatacggaacaatattacattttaaaactcagtccatatcaaacaacatcacaaaaatagataaggacaatgtgacaaactaatcacccctgccctacattttaatatttgcagtgtacaattaacggcatgcgtcacgcccttagacttttgtgtgaatttacaagtattttattcctcaattatatccatcaatttatatggttaacatttatttatttattttgggtgcaaattcacatggtttacttaatggcacagtttcttgaattataaacaaattcatgttacccctgttccaatatcgtctgcactaaaacagacaaaaaaaaatgtttactcgcatatattaggcgcggcccttccttgaatctttacacagatactttgtgtatcagactgtcttttacttgcacacgttattttcgtcaaatcaatgagtgtaatgcatgcgtattcaatataaactttgtactcccttccgtcctatttagttatactttggctaaaaatagttgttttaaaataatcatggtttaaaaaaaaaacaagaaagagttacttatattttttgcaattttaccctttctactctaataaatgttcctcaaagaagtaaaagagattaaggggagaaattaaaaaatagccagatttataagtggtcattctaaaatagtcacagtttcaaaagtaattgaaatttagtcacttttcatgtaaagataaatttgaacgaaaacattgttcaaaatccgaaaaaatacttcaatataatatactggaattccagtataatataccggtccagtatattatactggaactttccgtgtgttggagttctaacataatatgttggaagttcatacacaggtgcaccgatctccagtacattatgctggaacttttcgtgttgcagcaaaataatgattatttttcaatgactttgcaaacgctggctatttttgaatgactagtccgaaaactggctagccggtgctatttttatgagattgagagatctaagaataaataagggcaattcaatcaaataactcatattagtaatgttttcttaaagtatgcgtgcaaaaggctaagtaggagagagtattgattaatcgtgattaagtgtatatgctatcacttaaatttgagactcttaaacttgaacttattaatttaatgtaaacatcaggtgcgagtaagtattttcatgttaacagacacagtctcccaaacacaaaaaaatggaatgacctgtgacaagctgctagcaaaacataggccctgctaacaccaaaagactgttaaagttaaacttattaatttaatataaatatcaggtacgaataagtattttcctaactacagccgtcgactagtcttcaaattgctagcaaaacataggccctaataacaccaaagttcctatattaagtgctatatattgtcactttattttgagacggttaaaattaaacttattaatttaatataaacatcaggtacgagtaagtattttcataactacagtcgtcgactagtcttcaaattgctagcaaaacataggccctaaaaacaccaaaattcctatctctctgtgtatatatatgtaaagcacatatctaattttgaaataaaacattcatagattagctttttcaa

SEQ ID NO: 11 - DNA, 2001 bp, Nicotiana sp.
taaaaactgagtatgtcaacatgaggatcaactggcagatatacttacaaaaggattgtgaagagctcaacatgtacatttgctgaacaagctagggttgaagaatctgtatcaaccatcagcttgagagggagtgttaatcaacatggttaccactagtttatttataaagtgtaaatgctaaaccatagctagtgagttagttaatagttagttgagtttgttataaatattagtcagctgtacagtttaacatagcttctctttcagaaatgaaaattgctcttctctcatttcctctcttctagattcttcttctccctccttctcttagctcagatctctcttatgacagctaacaataaatacgaatatttcttgtaacggttgctcattgaatgttgtctttctcaaccgatatctttctttcaagttttccccccgattcgagtatttttgaaactcactcagcaccggtcacatattcgtaatcggtgccagctatttgcttactcatatcttatttgacttcattgtcacgtgtcagacagaagtatgtgcgcatataccatcaagtctcaatttgaaataaaatcaacttaagcagttaaaagtcaaatctcttttagttcggtctttaaaataataatttaaataatgaacctataaaacacgcaactcacactgaatataggggcagacataaaagccgaaagactgaattccgaaccggaccgaattatttcggtatttcgatatcggtttattcagtatttcggtactatttcggtataggatttttagttattcggtatttcggtacgatcctcggtattgaaatttcgatatttcggtataccgaaataccgaataatttaagtacaccttccttcactgcccagcccgttatcaattttcagcccaagtttctaacttgttatttctttcccttagccagtagcctactaagattaagcccaacgccccaacctaacattagaaattattataattagaaaagtataaagaaagtactcacattctactgctatgctcatgtagtgatttctattagaaattattagaagtgaaggtactgcccacattttcttgttgctatactcattatcacgcaattagaaattttctaatgaattagaattcagtagttcagcacagaggcggatgtagcgtattacctacgggttcaactgaacctataactttcgacacagagtaaaaatttatatgtaaaaattctttaaaattgtaaaaatcgtagatatgaacccataactttaaaaatataatgggtaacattaaaattgaacccatagaatttaaatcctggattcgcctctggttcagcattgtttagttcacaaaaatatggtacgatgccgaaccgtatcgaaaccataccgaaccaaacaagaagatatcgaacaataccgaactactttggtacagtatttggtatgcacacttgatatatcgaataccgaaataccgaaccgtaattttcgaataccgtaccgaaataccgaacactcacccataactaaacattaaaaagctagaactcaggtgtttaatgactaaacggaagtaagatctagataatccgtcactctgttgatttgtaaggctatcgacatgcaaaagtggaagcaaaatggagccgaaattttaacaaaaatgctgaaccaataccatgaaattgatgaatggtgggaccctatttcactcttttagaatttgcgtaagaccagaaaataacttcaatcgaaatcaaaataaataccaacccttttaggccccaaatcactacgtgtgatttgcaaacgtcattagccttatgtaaacagtgacctcatgccaacatattatcgcagcctataaatcttagtttacatttcattttctttcaaacacacacacctcacaatagaactaagttgtaagagtttcattttctttgttctttctcacaaaccaaaa

SEQ ID NO: 12 - DNA, 2001 bp, Nicotiana sp.
ttaactaccagaaatcacataaatacataaaatcaaaagtctatcacggaatatcaataaaaagagaaacataaaatgacaataagtaacaatttcaatttgaaacttatcaaataaatcttacttgttacttttcaaatgagtgaaaaaatcgaatcatgccagattaatatatgttaagacaaaacttaaagtaggaagattttgaatttttatagtttaactttaaatattttgcaccaatgcaagcttaacgcaagatactgctcatactattttcttttctgtttttgtaatgaagaatgatttttcttgcataaagattcttatctttttcgtgcatttgacgggattttttatttcttttttctttttctgtcaacaagaaatttatttttgttgtttcgtaacattttttcgatggcttgaaaccgaaaaactaaatcgattaaaccgaaccgaacatgaataaatcgaattgaaccgaaattattatggttcgattttgattattaaaatcacaaaccaaaaatcgaataaaccgaacctaacttctacaaaatcgaacagaaccgaccgacgcttacctgctcatttgtcaggtgagacaaatattaagtagccatcagaagatcattatatatatatatatggaatctctattgtgactccacctgtctcattttttaagtaggatttttattcaacttggtagaaaaagttaaatcgttactaattgacctatgtgttcatataaaaaattctaatatgtggtcgaaatttcaaagaccggcgcaagcgtcaagataaattaccaatggcaataagttgagtcttgaaatttgcaaacaatcacaacttgtattagcttcgactgagaaaaaaaatggaagaccaagtgaaactgctaggagcttttccaagtccctttagttatagggtaatttgggctctgaaacacaagggtatcaactatgaatacatagaggaagatctttcaaataagagccatgatcttttgacatacaaccctatctataagatgattcctgttcttgtacatgctggaaaaccaatagcagagtccacagtcatccttgaatacatcgaagagacatggcctcagaatcctttgctaccaaaggatcctcatgaaagggctcaggctagattctggatcaagttcggagaagataaggtaagttaatcatgttagtatgtttactttaggtccagtgtttgccaagagtttttaaatctaaatatcagaaggaaattaatgtagagtacttctagctagcattaaaatatttttactgaggattcatataattggccccaacttggtagtacatgctagttattgtcaagtgttaaatcgagtaaattacctcatctaaaattttaagcgctaaatgaaggatactatactttatttataataggtctgcgacacaccatcacttgcaggcttaattcatttttcttgagccaaaaacatgaaaattttgttcatatgtcacaacaatataatgagacttgaagaactcagctcttatattattagacatggatcaaatttacttagttattataggcctgtaacaacaagtaacatgttatatctttttaatatagagcccagaatttttcgcaatatttcacaagataggggaagagcaagtcaaggcaactgaaaaagcaaaggaagtgttgaaaattatagaagagcaaggtcttggagagaagaagttttttagcggggacacaattggattaagtgacatagtctttggatggatagcgttatggctggaagtcatacaagaagctgctgaagtaaaggtcttcgactcagttagtacttttcctcgtttacatgcttggatacataactttaagcaactccctgtaatcaaacaaaataccccacatcgggatgcaatgctagcttatttcaaacgtcgtcgagaaatggttgtagcagcggcacaaggttga

SEQ ID NO: 13 - DNA, 2001 bp, Nicotiana sp.
atcagtcctagcctcgaacgacttcgaagaacgttgtcagacaatcgagcatagccaacaaaaagccgaaatatccgtgaccaaccgaatattacggctggaatctcggcatgtatcgataaggaaccaacaatcagcgaatcagaagattttttacctttttatagagttgtaccaaaaataggactcttctactatataaagggggtctaatcattcatttgacatattgtaacacgcactcataagcaatacattattatttttatccgtcttttaagttcttgttctttttcatccataccggtctttgtgagttcggttcgagagtgactatttcacttaggctgaaactatccaactcttgtggtttaaatttatttggtctttgtttattcaatagaaacttaatttattgctttgtatcaagttaatccgcgtatccttaaaaccacttataaatttaattgttatccgattttgagggtaaacacctatatctatcattctattgtaatagttgatagggtttattatcaataaaacctcctagtttaatttagctgttccttcttctcttccaaatatttcactgttccattgcagctgcatcagataactaaggagaacaatttggatggtaggcccagagaaagatatgatctaagactagagagaaattcaccaagaaaatcgtactccttattaaaattttgtttaaacggtcaaagtagtacttctcgtcatcctaaatcctagtactatttaatggcggcttttatgtttctggaaaaaagtagttgcaaggagaaattaatttatggatgctgcgtttaactatagattggtgttaaacaatatcaaaactcaaaaaggttagcttcaaactaaataatatttagacattaattattatcctgtaatatttaaaattttcatcagaatactttccaatttgctaatattattattaattctaatatatatgctttttttttttgagaaatagagaaatatttattttctacgaaagatgactttcgtcttcttccgccaaaatataggtgaaaaatcgaagacgtccatagcagataaaatagagggcactcctacttgtagtaattgatcacacttaacatgaaagagctataatgttagttattcgttcggacgaactcgataatttttgtttaacttgtattagaaaatttattaaatatatataaatattttaattacagactcattaacttaaaagaagatatagactcattaacttaaaagaagatatagattccaacacaagttcaaaattcataaacgtcaaatcttggctaaatttctgaacatgaatgcattcctttaaaatatagataataagttaggatgttgtcactttcttaaagcatattccgactgagtctggtagaatctcataaactttaggccttatctcttcaattaggcaattacttacctccgctctactttaagaaaattcaatggagtacaccattattaagttcatataaaaataaaattatattaattctgtctcttgttggttcgctctatctttttctgttttcctgcttcaaccataacatatacaagaactacattttccaagctagatatatctaacatgactgactttgtaaatttcttttgccaagttaaagaaaaaaaatgatgttatccaaataataaagagaaagagccctaatgaaaaaaatgatttactattagagttgttcagctaatcacatcaattatggttttcatcaagtatgactaatggcggctcttatctcacgtgatgtgacattgaaattctttgactttaacactaatgtcatatgctttcaaattaataatccgataaagtctgctaacatgtgactttccaatttttttcttttacaaattgcagacttttcaactcttattccctattaaaacccatccatactattccttgtttctcaccaaaacccaaaa

SEQ ID NO: 14 - DNA, 2001 bp, Nicotiana sp.
tttcaaattactaagttgctaaaataaatacggctaataagtaccattatttacatgagtaaatactaaaagaaaaataagattcattttatctaaactatggaaaaactaaaaaatagatatccaacactgttttcattcatagtacaattgaattgaatgtcttttaatttattagtattagtatggatttgattttggtttagaatttatttgagttactaacatttatggactataaaacttattggagcatccaaaaattataagttccaacttgaaataatacattagaagataaaactatgaaaaaacttaagaaatatttataaactacactacaataaatatttttatgtagtaaatatatttaaaacttctatacttataatgtcgggtttgtttgatttcggtttgactttttttagttagaaccaaatcaaaccaaaccatagtcgggtttttttctcggtttggcgcggatttccgggttgatgcgatttgtcgatttcgtttgtacacccctaaatattacaatagattttttaaattggcagcatatataagttaatttcttaagttttgtatccctcagtataaagaatttattacactatcgggacatctttcctattatagcagaatttttttcttgtttcaaaattaaaaatctcacattttaagtaggcttgcccataattatttgggtgacctaatagtataagaaattcttcacattgacgagtattgaacttaaaactcttttattataaatttaaccttgatgccgttccatttaccgactcttcaaaccacatgaccagaatcaattctggaatccttcatcactaatcaatatctgttcgagggcatctcatagtcaaaatgtcgtagcaatatcataaaggaatgggaaaaaaaaatgaaaataaatcgcctctggtcgaagctcataatgaaaatttcggccccgcaaactttatcaagttctgctctcaggggttattttggtttgaggtataaaaagatttgatctcggtataaaatgtcgtatattacttatataatgtttggtttctattataaaattcttcccataactaatatagatgtctaataacaaatgctaatttccgaaaggaatatcggtcggaattcctcggaaattggctcgtcggtaacgtcgctaccagattttccatcgaaaatccctcctcgatgagccaatttccaatgggacattcgtcggaaatttacgtttttggtagaacttataactaatactacacaaattttggtttccacctatctaaagacaaaaatgccttaaataaggcagtcttacacaatgcttcaagcattattctacaacaattcatgcattattaatattcactcttgtattattattcccgatccatgcatgtattgtaattacggcatagctagacgcgcgggaaaccaaattaacgacctctaaacaacaataacaacccagtagaatctcaccggtggagtttggggagggtagagcgtacgcagaccttacccctatctcggaggtatagagagactgtttccgtgattgacgacgacctttaaattatttgtttatgaggtttgattaacttggacaagattgtttgtattcatattttaggcttcagttcacttaattaaactacctatatgagaacatcacatgaagtactaatactaagagaaaagactcaatgtaaggcggcttttaaacaattctcacgtttaactgtctcattcacaaaattagactgacttgtattatttcttttataagttcaactttttgcgtattcagaaagattctttaatttggccaactggctactatagggactcttttcttccagttatataatccttgtctctcaaattcaagatttgtaaaccaattcgttatccctttcttcaactttaacttctatatacttgagattttatctctatatatagctaaataaa

SEQ ID NO: 15 - DNA, 2001 bp, Nicotiana sp.
actatactatagtgtgatgatccaattggtcatttttgagatctaaaatttcttttctctatttgagacctctcatatgttcattagtaatatatgaattgtgggtatggtggcacgggttccgagggatttgaagccttatggaacacttgaactagaacttaaagccttaaattacgagaattgaccaaagttaatattttgagtaaacaaacttagattcatgatttgaaagtttcattaggttcgtatgacaattttggacttaattatatgttcaaagtaggatccgaggggttagggtataattcgacactatccaaaaaagttgtaaacttatgagttcataaattggatttgaactttaattttgagttgtgatgtttctatatatgttttgaacccttgaacaagttcgtatagaatatttaggcaagattcaaagtccaaattggactcgactaaattcagacttcttagctataactaagtaaattgtgttcttttgcgtggaaaaagtataacaccccatgcaagacaaaagtttgtaattcctcggtcttaatttatgtagcagtaatagattcagcatcgagtataaaaagaaaataaatttttgaaatttatgatctaaagtaagccatatacgtttgcgtaattacaaaccatctcattaagataaaataaaaagtttaaagttaaaatatttttaaataaaaaaatatgtcattctttttagataagctaattaaagaaaagtatatcagataaaatggaacaaaggaataccaagattaattgatctactttcaaattcaagtattacctcagctcaacaagaataattttttttggggggtaagtaattaatttggtatttgtttagactttacccttaccttttgtgagctaaagaggctggttccaatagaccgtcgatttaaaaaagccttttcaaaagaggtttgtaaaatacaggaattaaaaaaagatgaaaatactaaaaaagaaaaaggaaaaatattataatagtagtaaagaaaccaaagcaaaagaagcaacaatagtaataaaattaaagagtaagatgatgatggtgatgacaatgataatactaataataataataataatgatgatgatgatgatgatgatgatgatgatgatgatgatgatgatgatgatgatgatgatgatgatggggagaaaagggagaagataaggtgatctaaactagactatgttcttccacagaaaagagagaaatcactcgacgacctactaacattctactctaatcctcgactttcatgctcttctatctcgggtcgtgtcctaggtaagttgaaaatgtggcatgtctaattacctctctccaattcttcttcggtctacctctactctccttagacctatcattgccaacctctcgcactagggcatccatgctcctcctctttacatactaaaagtatcccagtcgcacttctcgcatcttgtcctccacagaggtcactcccactctgtcgtgaatatctttgttcctattcttatctctcctaatatgtccgccatatcacctgaaattacttaattttgtcatctgtcactcaccatttaattttttaaaaggtccaaatttaccccgatcaacttttgagtatagttcagaattacaagctagaaaaataatagtattaaatcaaagtctacggaggacgaagttgctcaatctcgcatgccgtatagtataggggcaacttcgccccttctccgaatattcgaccattttttctcataaaattctatgtctctccatcacaacatcagatttgaactttctacattttttttttcttcacttgtgacaaaaaatacactgttttaattccatgacgtgcttcactgggtgtgactttggctttttaagtctttgtcggtcatcttctgcttgtctatataagaagcagcctaatggttccttaaacacacaatttcagc

SEQ ID NO: 16 - DNA, 2001 bp, Nicotiana sp.
ttatgtgacattttttttctttttatgatgtttaaaaaaactagtatctcattaattaattaattatatgtctgaaaatattaatttttttactttaaactttctattctatctttagtgttatgatttttatatataaccatggaaatgccatgacttatttagtatcacgcgttttaaaaatttttcttttattttttaaaatttcatatattccagtcaaatagattcacataaaatgagacggatggggtaaatagtaaatcttaaagctagcaaactatgttcaacatcatttgatgggtttcttttttcaggataatattttatgtgtatttggtctttttggattgttttattaaaagaaaaactccttgagatgcatggtaagccaattgatcgtcattgttattttgaaataacaagtaccatatcatatgaggccgtgattatctaaagacagataaggaaattgggctatcaaaataaatatgtaagagttatgttcctcatcattaagtatgtgaaacaaaattgtcaacttgtacaacgattctggaatctacttggcgttttcaaagctctctgagccacaacaagttcttgcaattaagttttataaataatttccatgtcctcatatttcactatcttccagatatcccataagactacgtacgacaaacggcaccataaatattaatcataacaggaagactaaactcaatttctaatttccctattaccagaaaaattagaacaaataacaagaagactgtgatactccatgaagaaaaccattaaaacattccgggttcttactagaatgtggagtaatatatgctttcctgttttggaaagtgctaaacccacaggctaaggtaagaaaagtagtcccacatgctagaagcttcataggccccgactattataagctactatacgttgcttgacaaaagtggaaatgcaaatcgaattctcaaacttgcatctcactttccagcctaggccacaaaataaaagacgccataaattaattagttcgtggatcaagaggtcacaatttggacaacagtaacaaggttccatgtcaatctcctagttaatggtgttcctttggatttccctatcccttttaattagctactccctccgtctcaaattatctgtcgtgatttctaaagttattgtctaaatttatttttcatattagtagttcaagactaaattaattatttcttttccattttacccttaatatgatattgttcttgaagatgaagataatacataaataggaagattatatatatcttaaaacataaataagggtaaaatagtccaaacctcttctcattaatattttcttaattaagtggcgtgtaaaaaagaaacacgacagataatttgaggggagaatatttgtaaagaaaaacaacaatttgcttctaaacagacccaaaaggaatgttagcccaatcctggtaaaacataaatgtcagcaagacagtgctatgtttaattatcagaaattaacagtactacttgcaatcggaacacgactattaaacaaacaaaggtattatctaccagtacatttctctttcattaaattcctgtggtcagacttagttactgcccctttgagaattcttgtcctactacttcatcctcaactttccgtccaatatattattctggtcatttgtttatttctgaaaagcttggaattacatatatacatcctagtccatttaattaagataaaatttcctcattctccctgacatcaatatgtgctaaaagtcgcccttgtcactcaccctagttcacactcgagctttgggattggcattctctccatttcattataaattcaagccaccacacaacacagagtcacagagctaaatatagcatatatatatatatatatatatatatatatacctccctgcatatcttcctcagagtcaaattaagcttcaagcaaaacaacca

SEQ ID NO: 17 - DNA, 2001 bp, Nicotiana sp.
cataatgtattttctcaaagaattatataatatgtgtatactattaaaatacattgtatatgatagtaatccacaagtataatataatctatatataccattaagatatactagtaatatattcatatataccatcatcattcatcatgtttttaataattatacaacataatgaataattaaatttaatatagtactacgtataagtgtaaaaatagaggtacaatcagttacttgaaggaggagtggaataagaaataaattgaagacaaaagttggattgaatagacgcaaaaggaaaggttttagggtgaggaaaatttataattgtacagtattcaaaaagaggagaaagtgagggttttagggtacacggaattaaataggggagagaaaattattgggaaacttcaaaagttgtggattaccattaattactaatcctattttaatgggattggtccaacattataggtttatgctagaaatataacgtagttaataagctgccatatttgttactccctccggtccacaatatgtgatcaatttaccttttgattttggtccaaaataagtgtttaaaatagcacggtctagccagttttcggactggtcattcaaaaatagccagcgtttaccaagtcaatgaaaaataaccactattttgctgcaacagagaccggtccaacataatatattggagtttggtgcacctgtgtatgaacttccagataatatactggagcaccggtgctccaaactccagtatattatgctagaccgatatattatactagaactccagtatattatgctggagtatttttccggattttgaacaatattttcgttaagatatatctttacatgaaaagtggctaaatttcgattacctttgaaactgtggctatttttgaatgaccacttgtaaatctggcaatttttgaatttctcccccatttatataatcaagaaaaaatttgatttttttttaaaattatccttatatacgtatccctaaaaagttttttactcctcacattaaattatgctgcaacatttaattaagggtaatttagtcacactaactatttttgtctagaatttatatttccttaatgggtgtgcccaaggtaaattgaccacttatactggaccggagagagtaattgcttgctgctactagaatttagtaaaattttcttaaatattgccaaatatgttttttccacgtgttaatttggacgaatccagtaaattttgcttaactttatatttgtattaaaaaaattagtaactatatataaatattttaattatggacccggtaactaaaacgaagatacaaattccaagacaaattcagaaatcataaacatcaaatcttgtttgtacctatgaatgcattccttaaaatatactacaagttagggtgttgtcactttcttgaagcatattccgactgagtcttgtagaatctcatgagcgttaggccttatcgcttcaattaggcaattacttacctcctctgtactttaagaaaattcaatgtagtacaccattattaagttcatttcataaataaaattaattctgtcacctctataacatataagaacgtatattttccaagctagatatatctaacatgaatgactttgtgaaattcttttgccaagttaaagaaaaaaaatggtgtccaaagaataaagagaaaaggcccctaataaaaaaataatttattaattagagttgttcaaacaatcacgtcaataatggttttcatcaagaatgactagtggcggctcttatctcgagcgatgtggcatgattttgactttaacactaatatcaaatgctttctatatcaattatcctatagagtctgctaacaagtaattcaattctttaatttcttttacaaattccagacttttcaagtcttcttccctattaaaacccacccactctattccttgtttctcaccaaaacccaaa

SEQ ID NO: 18 - DNA, 2001 bp, Nicotiana sp.
atgaacgggtcgattttagggtatttgacatttaatcctctcggtctcacggtaggcattcggatcgatatttaaggaaaataaaatataaacaaactaatatatatatatatatatatatacacgacaccttaagatattagaagttggccaagaaatttaaatgaacaataacaaaagatttgctttttgcatctcgttgtccatgagattttctttgtctgctcacgacatttccaccttaaccatctaaatcaaaagttaatttgttcctacaatacgatatcgcaatcttattacgccctccattgcattttatggaaggtattattttttgtggagttatactattttttctttagttataattttcttatttttttttaaaaaaacattttgaatcattagctatgtagtactgttcgtgtaatttataaatatatataaaaaaatttaaaaaaatgaggaattaatagtaaattcacatcgaaaatcaagtgttttgactatcctactccacaccctgtcacataaattaggaaaaagaaagaaaaaaagaaaagaaaagaaataccttccaatttactgcttccctttaagaacatgaaaaatcttgctaatagattgctagtagttgttttctaaataactcacgtctctatcttgtctgccaccttgaaaatatatgactgtttctatcttttctttagataataatagttgagcaatcaatatctaaaactgtttttttctttcatcttaatctaatcattaagtaatcaatgtatttttaaccagtgctttatttttgctttgggtaagattgtttcatctatataacatttgttcctcaccaattactaccattaaacatgaacaaaatgtttcatggacagtgcattcttttcccttataaatcacgtatctatctatttctccaccttaaatccatatatatatatatatatatatatatatatatatatgtttcatggacagtgcattcttttcccttataaatcacgtatctatctatttctccaccttaaatccatatatatatatatatatatatatatatatatatatatatatatatatatatatatatatatatatatatatatatatacttttaatattgtatcctattaaggatcaatattttttcttctcgttttctgcgttgagtaaggtattaggtagattggttttaaagttgtacctccctcttaactcctcgtctttaataacgttaaatttagactgcttgacttatctcatgaataatgcaacgtgttccatataattcagatctccatctcttttactaccttgaatatatataatattgttatgaagttaaactaaaagaacaaaaaaatatagagagaaataacaacttttaaataacaataatagtaaaactaattcatacattgtgagacttgatctcttatgaaagtctcaaactttacagtaaaatgaaggaaaactaccggttatatccatttataagtatataattataaaaattggtgaattcataaaatattattaatattagtcaattagctatttgtaacccaaaaaaggttaaagttttgcttttatttgagtgtgtattattagaatagattaagtacattttaagaagcttgaatttcagttttgggatgatttggtggagttttaaggtggtttgaattaaaaattaaaagtagaagatgattaaaatttcatggtaaaggacaacagtaacttagcaagaccttatacacgtaatgagctaacactaatcttccatctccaataatgaaaatcatgagtttcgtggatcacgttttatactagcttttcatgcagctaactagaacataatatattatttaataataataaaaaactagaatataatctatataaagactacagcctctcagcactttctcaccacttccttttcaatacttactttctactatattgaagaagaaaata

SEQ ID NO: 19 - DNA, 2001 bp, Nicotiana sp.
ataaagtaaaaatgataaagttgaagaacaattgttgagcacggcaaacgagaaaagcagagtagaatattctattgaagtaaataataatgtgtttacaaatgattggggtcccctttatataggagggaaaaaccctaatatggtacattcccaactatggtgaagaattctattggtattgttgtataacaacctagtacggactcgtactattttgtacaaatcttatcccataatttatgccttgatccacgtgttcttgagaaattcccgctctttcttgagtgtcatcgaaattgtactgcccttgaggcagatcatgacgggtctccgattttctcctcgaggtgcgcacatcctggccagggtcgattcttacttcgagcttcccgaactcgagctcggggtatgatcaagccttcgaaatcgagctctccaatttcgaccgtatacaattttaagaattgaatatactttgatcttttcttgaaaaagtatttatttattttatcttctcgcctagcgcaatgaaatcaatatttattattttcaaaaacttacatttttctttagttttattttaataatatttttatattttttctaaaattatattcttattaatataggtacacgcgcagagcgcataccttaatactagcttgagggtacgtgttttgcatgtgtatcccatattctatatctatatctatactatattaaaaacactaacgctcttggcgaaatgccgttcgcttattttatccttaaaaaatattatatattggatatattatcctttaacatatataatcatcttcaggaacttatatttttattttattatttaaatataaatttttaataaattagtactcattgagatagaatacacgcgcatcgcgcgtaccttgaggctagtagaaaagaaaagtatgatagtatatgagtaacgtgttggaaattaagggaaggaaagaaaattttctttacatccaaatttgaaagttatttgacgtcatcgagatgacggccatgttcaagttttccacaaataatgtgaaaagaaaaagaagaagacacacactgtgtttggttttattatagttttttcttttagagaattgattgtacaaattattataagaaatagtataatataagatttagaaataagattattagaaaaaacaaacatcaaaaagtatttattttaatttctttttccaatggacattcccattcttctgaaacaacatagataaaaatatgaaagcaaaaattatcagatcgtttaatgcagataatattaattaacacattaaccataaccaatattttatttaaaaaaagcacaactgctagatcaaaaaagtgtttaacttcatgcattgacaattttttaaaataattttgcagcatcaggtaaaatattttttcttcgtttcccaccctgtgtacggtatacacgggtacttatattggggcccaactaaattcggattcgtccggagaagtcccacattggggcataaagcgctccctgacgaaggcgactccatacccatggacttgaacccgagacctttggttaaggatgaacgagacctccggtgccaggtaaaatattggtaactgcttatataagtttaatatggtaacctgagccgaaggtctatcggaaacagactttctgccctatcagggtaggggtaaggtctgcatacacagtaccctctccaaaccccacttagtgagactttagtgggtagttgttgttgttattgttatggtaacctgggaaacaggataaataactatctataacaggatatattacattgatattaccatgtcaaaaaattaagcaagtacatgaataatcgccgtgaaatcttcaagatttctcctataaatacccttggtagtaaatctagtttttccattcaaagtacaacatttctcctatagtcatggaatttgttctcttttcacaaa

SEQ ID NO: 20 - DNA, 2001 bp, Nicotiana sp.
aaatttttgctaaagtactctctttttattagttgaaaaagaaattactctttctataacatgaaaataaagtactcatttgttgaaatgaaagaaaatatttttttctacatcatgaaaagatactcgttatggggacatggcgaataggggtgggttggtggggatatggggaatagggggaagattgaaaaagagttttgggaaagtttttttttgttttgatagggaaaatattttcctccaatttgagaaaaatgagttcatgggcgtggggtggaggtgggtagctggaggtgtggggtgggttggtggggatatgtggaataggggaagattggaaaagagttttgggaaagtatttttttttgttttgatggggaaaacattttcctctaattgatgaaaaatgagttcactagaaaaatattttccaaaatatttaatccaaccaaacatgataaaattaaaaaatatttaaaaatattttcgttcgtaccaaacacacccacagtggaactgattaatctgtgtgttacgtaatttgtgccgcttcatgcatttatttcgtgcgacgatttggaattcttcaataaataactaatagtgaaagatcatataatactagtaatactagctttaaaaaaatgtaagtgtcgggagggtgacggaaatgacaattatgtcataaacacacgttgttcatacttcacataggggcgactctaaggctttgggaccataatagtagcagcagtagtaatagtagtcgtaatcatagtaacagtagtggtaataatcgtagtggtgatagtggtggtaatggtagtgatggtagtggtagtaataatagtagcagtagtgatagtaataataatagtaatagtagatagtggtggtagtggtagtagtaatagtggtagtagatattcaccaataagcgtgctacttaatagaataaactacaacaatcgtttaaattgatcaggagtaaatacttttgacaccgtcaatactcaaaacttaagctattacgttatatatgtacgcttattctttttctcgtttgtgatgatagccaaatcaaaattttcaatttgagttctagacctcgacattcgatagtccaccactttattttttgtgctctttttcctaatttgtttttgaaattcgcttttttgtcttaaatgatttaaaagtaaattttattgttagtgtaaatattttataaaataaatttaagagcctctcaatatgatttcatcttaggccacgaaatccgttgagcacaggggcggagccaccttatgggatgcgtgacaccgcttcatcggaaagatttattaaatacatatatagacatatgcaaaaccaaataatacataaaaacgataaaggtgacaacacttgaaataaaataactcattgtccaactggttaagcgtttcaacttcttagtatgtcgggagtacgaatccttttggtggaacccttatgtttttattgttttgaagacattatttattaaaaaagaattaaaatatattctatattagtaaggacctctaacaaaattaagcaacaacaaaagtcacttgaacaagaattcatttgttagtcaatttgacaataaatatactcaaatcattcttggaaaaagacatatttggtactagtatttctaacaagattattattaatacatttagaaaataaaaactcgttgtaaagatttatagtaatgttttgaattttattttttttaataaatacaatgtcattatagttattcatttgttcacttctttgtttacctattacaaaatatgatacggacttacgaaaaattttgcgtacgacactggttgagctgcccctgtgttcacattggaagaataatatcatggcacatttcttctctataaattcaaggttagcatggtcgaataaagcatccaaaacaaatatcgcatatccaatctaaagaaacaaaaaaaa

SEQ ID NO: 21 - DNA, 2001 bp, Nicotiana sp.
aagggaaaaaaataaaaatagaagagaaatgcaagggtttgctttcttgtaccaaatattgaaagaaaaaaaatgttacaaccatttcatttgcaaaaaaaaaaaataaaaaaataaattgaaattgaaattcaaaagtaaagctgtttggttcggaacagaagtcgattttgaaaatcgaaccgacgcgttttacgaaaatgaaaacgaccatcgctagattttcacaaactaaaacaattttttccagaaaccttatacccataagcaaattcaacacataaattctccccaattatttttaagaaaatttagaactattttttaagaaattaaattaaaccaactcaactattcaagcaacgcattaagtataacggattcttaaagtctcgttcttaattctcgaaatgtgtcgagaaatcacaaccgttaaatctaatgcctcaaagtaaagaaaatgaataaggagtgtagcaaaaatatcaatgtggacaagatggtcgtatataatttgtacaaagaaaattcaaatgggaatctcttacccagtcaaaacatgcatattctcttggattctaggcaagctttcccattccaaagtcaatggaacgaaccaattattgctctctaagtctttttctttcactaaagagtaaattcaatatcttgacaattaggcactaagtaaactgaagaaatagaatcccaatatttttccttcctcgtaacaataacattaaagactcatcaatgtgactcgaccaaaggttcagtagcttcattttcacaaataggggtgacaatttgaatccaaatccatctagcccgtccaaagattaatggttgagctacaaacattttaatttatgagttaatttaggctgagcccaagttaactcattatttttttataactcattctgacccattaaacagcccaaatataactcatgaaactcacgcaaaacaaagaatctcagtccaatttatctagaaatttacttaatcaccccaatttcacttttttttttgtatttttaattttctgttcttttatttttctgcaccacccaccctacccctatcccccccaaaccccctcaaaaattaatttttacctttttttttttttaatattttcaatttttttttttgtatttctgcaccacccacccgccctaaccccctacccccggcaaaaaccctcaattttttttactttttttgtttattttttttaattttttattttttttttatttttctacaccaccctaaaagtatagtacaaaattcagatttgaactcctttttattggtagattaatcaaagtagaaaaaaaaagacagtttgaaaactacctcattctataaggttttcagaactcgtttgcttactgagaaaatgaattattcacagttaaaatatattttaatgttcaatataagtaatatcagcataatttttataccacatctaacgagggataacaattcagggattagctataccggaataaaacaagtaaaatgataaaattgtccttctaccaaagccttttaaaggaaaatcaaggttaatattagaaacaaaacattatcaaagttaatttagtttaaaaccaaataaatgctttatacgtatatcttattactaatgcagtaaaccaaataaatcagaggtactaaatgatctcaatattagtacaatttagttacgtactaaaatttctaacataattttattctcgccaaccctacaagtatagtactccaacccctttctcttggcaaaataatccaataggaaataaagacggtaagaaaattggcacacgttatatatgacttttgacactatttaagccagccaatggcattagtggttgcatactttgaatgtagagaaataactaataaagactgttgagagttgtttcttcttaccccttttgaagtttattttcctcagattttcacagttccaagcaagcacta

SEQ ID NO: 22 - DNA, 847 bp, Artificial Sequence
  Description of Artificial Sequence: Synthetic polynucleotide
gccattcttcagtccacaataggcggcggagcttcacctacagcggcggcggcggaaaacggtaccagaaaagtcatccctctctcaagagatgccctccaagatttcatgttatcaatcataacccaaaaattacaagatgagaaacaacctttttacgtgttagatttgggtgaagttgtttctcttatggaccaatggaaatctgctctcccaaatatccgtccattttacgctgttaaatgtaaccctgaaccgtcgttcctttcaattttatctgctatgggctcaaattttgattgtgctagccgagctgaaattgagtacgttttgtcccttggcatttctaataagatcttcaacacctacaccatttttttaatcactactacccattgcattgaacaaacttccaagttcttcttagcttcagattaagaaagtaccctttcttggctttgttgatgtggtaccattgtccattgtcttgtgtgtttccagaaatgccaagggacaaaacgtactcaatttcagctcggctagcacaatcaaaatttgagcccatagcagataaaattgaaaggaacgacggttcagggttacatttaacagcgtaaaatggacggatatttgggagagcagatttccattggtccataagagaaacaacttcacccaaatctaacacgtaaaaaggttgtttctcatcttgtaatttttgggttatgattgataacatgaaatcttggagggcatctcttgagagagggatgacttttctggtaccgttttccgccgccgccgctgtaggtgaagctccgccgcctattgtggactgaagaatggc

SEQ ID NO: 23 - DNA, 1302 bp, Nicotiana sp.
atggccggccaaacaatcatcgtttccgggttgaacccggcggccattcttcagtccacaattggcggcggagcttctcctacagcggcggcggcggcggaaaacggcaccagaaaagtcatccctctctcaagagatgccttacaagatttcatgttatcaatcataacccaaaaattacaagatgagaaacaacctttttacgtgctagacttgggtgaggttgtttctcttatggaccaatggaaatctgctctcccaaatatccgtccattttacgctgttaaatgtaaccctgaaccgtcgttcctttcaattttatctgctatgggctcaaattttgattgtgctagccgagctgaaattgagtatgttttatctcttggcatttcacctgaccgtattgttttcgcaaatccatgcaaaccggaatccgatattatttttgcagcaaaagttggggtgaatcttacaacctatgattctgaagacgaggtttacaagatccgaaagcatcacccgaaatccgaactcttgctccgcatcaagcccatgctcgacggcaacgcgagatgcccaatgggcccgaaatacggcgcgcttccagaagaagtcgacccgctgctccgggcagctcaagccgcccgtctcaccgtatccggcgtctcattccacatcggtagcggagatgccgattcaaacgcttatctcggcgccatagccgcggctaaggaagtgtttgaaacagctgctaaactcgggatgtcgaaaatgactgttctagacgtcggcggcgggtttacatccggccaccagttcacaaccgccgccgtcgccgttaaatcagctttaaaacaacacttcgatgacgaaccggagttgacaatcatagctgaaccgggtcggttttttgcagagacggcgtttactttggcaacgacgattatagggaaaagagtgaggggtgaattgagggagtattggattaacgacgggctgtacggttcgatgaactgtgtactttacgaccatgcgacggtgaatgcaacgccgttagctgttctgtcgaatcgtagtaacgttacctgcggcgggtcgaaaacgtttccgacgactgtgtttgggcccacttgtgatgctcttgatactgttttaagggattaccagttaccggagctgcaggttaatgattggctggtttttcctaatatgggtgcttatactaaagctgctgggtccaattttaatggatttaatacttccgccattgttactcacctcgcttattcttatccaagctga

SEQ ID NO: 24 - DNA, 1299 bp, Nicotiana sp.
atggccggccaaacaataatcgtttccgggttgaacccggcggccattcttcagtccacaataggcggcggagcttcacctacagcggcggcggcggaaaacggtaccagaaaagtcatccctctctcaagagatgccctccaagatttcatgttatcaatcataacccaaaaattacaagatgagaaacaacctttttacgtgttagatttgggtgaagttgtttctcttatggaccaatggaaatctgctctcccaaatatccgtccattttacgctgttaaatgtaaccctgaaccgtcgttcctttcaattttatctgctatgggctcaaattttgattgtgctagccgagctgaaattgagtacgttttgtcccttggcatttcacctgaccgtattgtttttgcaaatccatgcaaaccggaatccgatattatttttgcagcaaaagttggggtgaatttaacaacgtacgattcagaagacgaggtttacaagatccgaaagcatcacccgaaatccgaactcttgctccgaatcaagccaatgttcgacggcaacgcgaggtgcccaatgggtccaaaatacggcgcgcttccagaagaagtcgagccgctgctccgggcagctcaggccgcccggctcaccgtctccggtgtctccttccacatcggcagcggagatgccgattcaaacgcttatctcggcgccatagccgcggctaaggaagtgtttgaaacagctgctaaactcggtatgtcgaaaatgactgttctagacgtcggcggcgggtttacatccggccaccagttcacaaccgccgccgtcgctgttagatcagctttaaaacaacacttcgatgatcaaccggagttgacaatcatagctgaaccgggccggttttttgcggagactgcgtttactttagcgacgacgattatagggaaaagagtgaggggagaattgagggagtattggattaacgacgggttgtacggttcgatgaactgtgtactttacgaccatgcgacggtgaatgcaacgccgttagctgttttgtcgaatcgtactaacgttacctgcggcgggtcgaaaacgtttccgacgactgtgtttgggcccacttgtgatgctcttgatactgttttaagggattaccagttaccggagctgcaggttaatgattggctagtttttcctaatatgggtgcttatactaaagctgctgggtccaattttaatggatttaatacgtccgccattgttactcacctcgcttatgcttatccaagctga

SEQ ID NO: 25 - DNA, 807 bp, Nicotiana sp.
atgccagatttaatccgttcaattgcagagaaccatgaagctggccagccattttatctcatggatttggctataattgaaaagctaatggacaaatggaaccattcttttccaaatataaaacctttctatgctgtgaaatgcaacaccgaacctgctcttcttactaaactagccaaattgggtgcaaattttgattgtgctagccaactagaaatagaaaccgtcttaaatctcgaaattggcccaaaccaaatcatatttgctaacccatgcaaagctatttcccacatcaaatacgcagccaatgttggggtcaatctcacaacttttgattccaaacttgaaattgacaagatcaagaaatggcacccacattgtcatttgttgcttcgagttaaagcgcctaatgatagcggcgcattacgtcccctgggaaaaaaattcggcgtgctaccagaagaagttgagccactactgcattacgcttgtaatgtggtcgggctaaaagttgtaggcgtttcatttcatgttggatctatagcacaaaatcctagcatttatcgcgaggcgattgcagctgctagggccgtttttgatgttgctgatcatcttcgaatgcctaaaatgcaaattttaaacattggtggaggatttagatcaacaccattgttcgaggaaatagctagtgtagtaaacgaggcagtccaagattattttcccatgactaatttaacaatatttgcagagccagggcggtttttttgcagaaacggaatttacgttagtcgctcatgtgattggtaa

SEQ ID NO: 26 - DNA, 1140 bp, Nicotiana sp.
atgccagatttaatccgttcaattgcagagaaccatgaagctggccagccattttatctcatggatttggctataattgaaaagctaatggacaaatggaaccattcttttccaaatataaaacctttctatgctgtgaaatgcaacagcgaacctgctcttcttactaaactagccaaattgggtgcaaattttgattgtgctagccaactagaaatagaaaccgtcttaaatctcggaattagcccaaaccaaatcatatttgctaacccatgcaaagctatttcccacatcaaatacgcagccaatgttagggtcaatctcacaacttttgattccaaacttgaaattgacaagatcaagaaacggcacccacattgtcatttgttgcttcgagttaaagcgcctaatgatagtggcgcattacgtcccctgggaaaaaaattcggcgtgctaccagaagaagttgagccactactgcattacgcttgtaatgtggtcgggctaaaagttgtaggcgtttcatttcatgttggatctatagcacaaaatcctagcatttatcgcgaggcgattgcagctgctagggccgtttttgatgttgctgatcatcttcgaatgcctaaaatgcaaattttaaacattggtggaggatttagatcaacaccattgttcgaggaaatagctagtgtagtaaacgaggcagtccaagattattttcccatgactaatttaacaatatttgcagagccagggcggttttttgcagaaacggcatttacgttagtcgctcatgtgattggtaaaagagttagaggtgagaaaatagaatattggattgatgaagggatttatggatcatttaggccaacactttataatagttgttttgtgggtataaagccattgttacttcaggtaacagaaaaatcttgtcaaatttatgagtcaactatttatggaccaagttgtgactcacttgatgcagtggctattgacataaacttgccggagcttcatttggatgacctgatagtgttttctaatatgggtgcatattcaacatgtggaggaactaagttcaatggatttgatatgttatctacacctgcctatcttgttaactcaaattctagctaa

SEQ ID NO: 27 - DNA, 1140 bp, Nicotiana sp.
atgccagatttaatccgttcaattgcagaaaaccatgaagctggccagccattttatctacttgatttggctataattgaaaagcttatggacaaatggaaccattcttttccaaatatgaaacctttctatgctgtgaaatgcaacactgaacctgcacttcttactaaactagccaaattgggtgcaaattttgattgtgctagccaactagaaatagaaaccgtcttaaatctcggaattagcccaaaccaaatcatatttgctaacccatgcaaagctatttcccacatcaaatacgcagccactgttggggtcaatctcacaacttttgattccaaacttgaaattgacaagatcaagaaatggcaaccacaatgtcatttgttgcttcgaattaaagcccctagtgatagtggcgcgttacgtcccctgggaaaaaaatttggtgtattaccagaagaagttgagccattactgcattatgcttataatgtggtagggctgaaagttgtaggcgtttcatttcacgttggatctatagcacaagatcccagcatttatcgcgaggcgattgcaactgctaggaccgtgtttgatgttgttgatcatcttcgaatgcctaaaatgcagattttaaacattggtggaggatttagatcaacaccattgttcgaggaaatagctagtgtggtaaatgaagcagtccaagattatttttccatgcctaatttaacaatatttgcagagccaggacggttttttgcggagacagcctttacattagtcactcatgtgattggtaaaagagttagaggtgaaaaaatagagtattggattgatgaagggatttatggatcatttaggccaacactttataatagttgttttgtgggtataaaaccattgttacgtcaggtaacagaaaaatcttgtcaaatttgtgagtcaactatttatggaccaagttgtgactcacttgatgcagtagctattgacataaaattgccagagcttcatttggatgacctgatagtgttttacaacatgggcgcatattcaatatgcggaggaactaaattcaatggatttgatatgttatctacacctacctatcttgttaacgcaaactctagctaa

SEQ ID NO: 28 - DNA, 1053 bp, Nicotiana sp.
atggacaaatggaaccattcttttccaaatataaaacctttctatgctgtgaaatgcaacagtgaacctgcacttcttactaaactagccaaattgggtgcaaattttgattgtgctagccaactagagatcgagaccgtcttaaatctcggaattagccccaaccaaatcatatttgctaacccatgcaaagctatttcccacattaaatacgcagccaatgttggggtcaatctcacaacttttgattcaaaacttgaaattgacaagatcaagaaatggcacccacaatgtcatttattgcttcgaattaaagcccctagtgatagtggctcgttacgtcccctgggaaaaaaattcggcgcgttaccagaagaagttgagccactactgcattacgcttgtaatatggtcgggctaaaagttgtaggcgtttcatttcacgttggatctatagcacaagatcccagcatttatcgcgaggcgattgcagctgctaggaccgtgtttgatgttgctgatcatcttcgaatgcctaaaatgcaaattttagacattggtggaggatttagatcgacaccattgttcgaggaaatagctagtgtagtaaaaaaagcagtccaagattatttacccttgcccaacttaacattatttgcagagccagggcggttttttgcagaaacggcctttactttagtcactcatgtgattggtaaaagagttagaggtgagaaaatagagtattggattgatgaagggatttatggatcatttaggccaacgctttacaatagttgttttgtgggtattaagccatttttacgtcaggttgaagaaaaatcttgtcaaatatgtgagtcaactatttatggaccaagttgtgactcacttgatgcagtggctattgacataaaattgcccgagcttcatttggatgatctgatagtgttttataacatgggcgcatattcaatatgtggaggaactaagttcaatggatttgatatgttatctacccctatctatcttgttaattcaaattcaagctaa

SEQ ID NO: 29 - protein, 433 aa, Nicotiana sp.
MAGQTIIVSGLNPAAILQSTIGGGASPTAAAAAENGTRKVIPLSRDALQDFMLSIITQKLQDEKQPFYVLDLGEVVSLMDQWKSALPNIRPFYAVKCNPEPSFLSILSAMGSNFDCASRAEIEYVLSLGISPDRIVFANPCKPESDIIFAAKVGVNLTTYDSEDEVYKIRKHHPKSELLLRIKPMLDGNARCPMGPKYGALPEEVDPLLRAAQAARLTVSGVSFHIGSGDADSNAYLGAIAAAKEVFETAAKLGMSKMTVLDVGGGFTSGHQFTTAAVAVKSALKQHFDDEPELTIIAEPGRFFAETAFTLATTIIGKRVRGELREYWINDGLYGSMNCVLYDHATVNATPLAVLSNRSNVTCGGSKTFPTTVFGPTCDALDTVLRDYQLPELQVNDWLVFPNMGAYTKAAGSNFNGFNTSAIVTHLAYSYPS

SEQ ID NO: 30 - protein, 432 aa, Nicotiana sp.
MAGQTIIVSGLNPAAILQSTIGGGASPTAAAAENGTRKVIPLSRDALQDFMLSIITQKLQDEKQPFYVLDLGEVVSLMDQWKSALPNIRPFYAVKCNPEPSFLSILSAMGSNFDCASRAEIEYVLSLGISPDRIVFANPCKPESDIIFAAKVGVNLTTYDSEDEVYKIRKHHPKSELLLRIKPMFDGNARCPMGPKYGALPEEVEPLLRAAQAARLTVSGVSFHIGSGDADSNAYLGAIAAAKEVFETAAKLGMSKMTVLDVGGGFTSGHQFTTAAVAVRSALKQHFDDQPELTIIAEPGRFFAETAFTLATTIIGKRVRGELREYWINDGLYGSMNCVLYDHATVNATPLAVLSNRTNVTCGGSKTFPTTVFGPTCDALDTVLRDYQLPELQVNDWLVFPNMGAYTKAAGSNFNGFNTSAIVTHLAYAYPS

SEQ ID NO: 31 - protein, 268 aa, Nicotiana sp.
MPDLIRSIAENHEAGQPFYLMDLAIIEKLMDKWNHSFPNIKPFYAVKCNTEPALLTKLAKLGANFDCASQLEIETVLNLEIGPNQIIFANPCKAISHIKYAANVGVNLTTFDSKLEIDKIKKWHPHCHLLLRVKAPNDSGALRPLGKKFGVLPEEVEPLLHYACNVVGLKVVGVSFHVGSIAQNPSIYREAIAAARAVFDVADHLRMPKMQILNIGGGFRSTPLFEEIASVVNEAVQDYFPMTNLTIFAEPGRFFCRNGIYVSRSCDW

SEQ ID NO: 32 - protein, 379 aa, Nicotiana sp.
MPDLIRSIAENHEAGQPFYLMDLAIIEKLMDKWNHSFPNIKPFYAVKCNSEPALLTKLAKLGANFDCASQLEIETVLNLGISPNQIIFANPCKAISHIKYAANVRVNLTTFDSKLEIDKIKKRHPHCHLLLRVKAPNDSGALRPLGKKFGVLPEEVEPLLHYACNVVGLKVVGVSFHVGSIAQNPSIYREAIAAARAVFDVADHLRMPKMQILNIGGGFRSTPLFEEIASVVNEAVQDYFPMTNLTIFAEPGRFFAETAFTLVAHVIGKRVRGEKIEYWIDEGIYGSFRPTLYNSCFVGIKPLLLQVTEKSCQIYESTIYGPSCDSLDAVAIDINLPELHLDDLIVFSNMGAYSTCGGTKFNGFDMLSTPAYLVNSNSS

SEQ ID NO: 33 - protein, 379 aa, Nicotiana sp.
MPDLIRSIAENHEAGQPFYLLDLAIIEKLMDKWNHSFPNMKPFYAVKCNTEPALLTKLAKLGANFDCASQLEIETVLNLGISPNQIIFANPCKAISHIKYAATVGVNLTTFDSKLEIDKIKKWQPQCHLLLRIKAPSDSGALRPLGKKFGVLPEEVEPLLHYAYNVVGLKVVGVSFHVGSIAQDPSIYREAIATARTVFDVVDHLRMPKMQILNIGGGFRSTPLFEEIASVVNEAVQDYFSMPNLTIFAEPGRFFAETAFTLVTHVIGKRVRGEKIEYWIDEGIYGSFRPTLYNSCFVGIKPLLRQVTEKSCQICESTIYGPSCDSLDAVAIDIKLPELHLDDLIVFYNMGAYSICGGTKFNGFDMLSTPTYLVNANSS

SEQ ID NO: 34 - protein, 350 aa, Nicotiana sp.
MDKWNHSFPNIKPFYAVKCNSEPALLTKLAKLGANFDCASQLEIETVLNLGISPNQIIFANPCKAISHIKYAANVGVNLTTFDSKLEIDKIKKWHPQCHLLLRIKAPSDSGSLRPLGKKFGALPEEVEPLLHYACNMVGLKVVGVSFHVGSIAQDPSIYREAIAAARTVFDVADHLRMPKMQILDIGGGFRSTPLFEEIASVVKKAVQDYLPLPNLTLFAEPGRFFAETAFTLVTHVIGKRVRGEKIEYWIDEGIYGSFRPTLYNSCFVGIKPFLRQVEEKSCQICESTIYGPSCDSLDAVAIDIKLPELHLDDLIVFYNMGAYSICGGTKFNGFDMLSTPIYLVNSNSS

SEQ ID NO: 35 - DNA, 22 bp, Artificial Sequence
  Description of Artificial Sequence: Synthetic oligonucleotide
ttggctaggagagtcagaagtg

SEQ ID NO: 36 - DNA, 22 bp, Artificial Sequence
  Description of Artificial Sequence: Synthetic oligonucleotide
tcatcgaacgcttgttcccgtg